European Patent Application EP 4 631 527 A1, published October 15, 2025. Title: Nanoparticle Comprising Peptide-based Conjugate for Delivering mRNA into B cell and T cell and Uses Thereof. Applicant: Seoul National University R&DB Foundation. The sequence listing filed with the application follows.

SEQUENCE LISTING (19 sequences)

SEQ ID NO: 1 - protein, 16 aa, synthetic construct
LKKLLKLLKKLLKLAG

SEQ ID NO: 2 - protein, 16 aa, synthetic construct
IKKLIKIIKKLIKLAG

SEQ ID NO: 3 - protein, 16 aa, synthetic construct
LRRLLRLLRRLLRLAG

SEQ ID NO: 4 - protein, 16 aa, synthetic construct
  SITE 9: note = Ornithine
  SITE 13: note = 2,3-diaminopropionic acid
LKKLLKLLXKLLXLAG

SEQ ID NO: 5 - protein, 16 aa, synthetic construct
  SITE 9: note = Ornithine
  SITE 13: note = 2,3-diaminopropionic acid
LRRLLRLLXRLLXLAG

SEQ ID NO: 6 - protein, 16 aa, synthetic construct
  SITE 9: note = Ornithine
  SITE 13: note = 2,3-diaminopropionic acid
LRKIIRLIXKLLXLAG

SEQ ID NO: 7 - protein, 16 aa, synthetic construct
  SITE 9: note = Ornithine
LKKLLKLLXKLLKLAG

SEQ ID NO: 8 - protein, 16 aa, synthetic construct
WKKLLKLLKKLLKLAG

SEQ ID NO: 9 - protein, 16 aa, synthetic construct
WRRLLRLLRRLLRLAG

SEQ ID NO: 10 - protein, 16 aa, synthetic construct
WRKLLRLLKKLLKLAG

SEQ ID NO: 11 - protein, 16 aa, synthetic construct
  SITE 6: note = 2,4-diaminobutyric acid
LKKLLXLLKKLLKWAG

SEQ ID NO: 12 - protein, 16 aa, synthetic construct
  SITE 6: note = 2,4-diaminobutyric acid
LRRLLXLLRRLLRWAG

SEQ ID NO: 13 - protein, 16 aa, synthetic construct
  SITE 6: note = 2,4-diaminobutyric acid
LKRLIXIIKKLIKWAG

SEQ ID NO: 14 - protein, 16 aa, synthetic construct
  SITE 9: note = Ornithine
  SITE 13: note = 2,3-diaminopropionic acid
LKKLLKWLXKLLXLAG

SEQ ID NO: 15 - protein, 16 aa, synthetic construct
  SITE 9: note = Ornithine
  SITE 13: note = 2,4-diaminobutyric acid
LRRLLRWLXRLLXLAG

SEQ ID NO: 16 - protein, 8 aa, synthetic construct
PLVFNQER

SEQ ID NO: 17 - protein, 12 aa, synthetic construct
HTHGAARVPDHR

SEQ ID NO: 18 - RNA, 1461 nt, synthetic construct
  source 1..1461: mol_type = other RNA
atggaagtccaattgttggaatctgggggtgggcttgtccaacctggtggttcactccgtctgagctgcgccgcttccggattcactttctccaccttttctatgaattgggttcgccaggccccaggcaagggacttgagtgggttagctatatcagcaggaccagtaaaaccatctactacgccgacagcgttaagggaaggttcactatatcccgggacaattctaagaatactttgtacttgcaaatgaactctttgcgggcagaagatactgctgtctactattgtgcacgaggtaggttttttgattattggggtcaggggaccctcgtaaccgtttccagtgggggcagcgagggtaagagctccggttcagggtcagaatctaaaagcactggtggctccgatatacaaatgacccagagtccaagctctctttcagccagcgtgggagacagggtgaccatcacctgtcgagcatctcaatccatttcatcatacctcaattggtatcaacagaagcctggggaagcaccaaagttgcttatttattctgccagcgtactgcaaagtggcgtaccttcccgcttctccgggtctgggagtggcactgattttaccctcacaattagcagcctgcaacccgaggacttcgctacatactactgccaacaaagtgtaatgatacccatgacattcgggcaaggcacaaaagtcgagataaagggaagtggaggaggtggctctatgccccgccgcgctgagaactgggatgaggccgaagttggtgctgaagaggccggagttgaagaatatgggccagaagaagatggcggtgaggaaagcggggctgaagagagcggtccagaggagtctggtccagaggaacttggagctgaggaggagatggaggccggacgtccacgtcctgtcctgcgatcagttaactcaagggagccctcacaggttatcttttgtaatcgaagccctcgcgtggttttgcccgtctggctcaacttcgatggtgaaccccaaccatacccaaccctcccccctggtaccgggcggaggattcattcctatcggggacacctttggctcttccgagacgctgggactcacgatggcctgttggtcaatcagaccgaactgtttgtgcccagcctgaacgtagacgggcagccaattttcgcaaacataacactgcccgtatatacattgaaagaaaggtgtcttcaggtggtacgcagtctggttaaaccagaaaactataggcgtctggatatcgtgcgcagcctctatgaggaccttgaagaccaccctaacgtgcaaaaggacctcgagcggctcactcaggagcgcatagctcatcagcgcatgggagatgaaaacctttactttcagggtgggagcggcggcagcggcgggagtcatcatcaccatcatcatcaccactga

SEQ ID NO: 19 - RNA, 1398 nt, synthetic construct
  source 1..1398: mol_type = other RNA
atggaagtgcaacttctcgaatctggaggggggttggtacaacccggcggcagcttgcgcttgtcctgtgctgccagtgggttcacattttctacattctctatgaactgggttagacaagcccctggcaaagggctggaatgggtgagctatataagtcgcacctccaaaactatttactatgcagatagtgtcaagggacgatttactatcagcagagataactctaagaacactctgtatctccagatgaattcccttcgagccgaagacaccgcagtatattactgtgctagagggcgcttcttcgactactgggggcaaggcactctggtaactgtcagtagcgggggttctgagggcaaaagttcaggatctgggtccgagtctaagtcaactggcgggagcgacatacaaatgactcagagccccagtagcctgagcgcctccgttggtgacagagtcactattacatgtcgggcatctcaatctatttcctcttatcttaactggtatcagcaaaagccaggcgaagcccccaaactcctgatatactccgctagtgttcttcagagtggcgttcctagtcgcttcagcggatccggaagtggcactgattttacacttacaattagttccttgcagcctgaagattttgccacatactactgtcagcaatcagtcatgattcccatgacctttgggcaagggaccaaagttgagatcaaaggctccggaggaggagggtctatggaaaacagatggcaagttatgatcgtttggcaagtagatcgtatgcgaatacgcacatggaaatcactggtaaagcaccacatgtatgtgtcaggcaaagcacgaggatggttttatcgtcatcactatgagtcaccacatccccgcatcagctctgaggtgcacataccactcggtgatgctcgtctggtcataactacctactggggcctccacactggtgaaagagattggcacctcggccaaggagtaagtatagaatggcgcaaaaagcgttattcaacccaagtggatcctgagttggcagatcagttgatccacttgtattactttgactgcttcagcgatagtgctattcggaaggccctcctcgggcacattgtaagcccacggtgcgagtatcaagctggtcataacaaggttggtagcctccagtacttggctttggctgcacttataacacccaaaaagataaaacctccactcccctcagtgactaaactcactgaggatcgttggaacaaaccccagaaaaccaaggggcacaggggttcacacaccatgaatggccacgagaatttgtatttccaagggggatccgggggcagtggagggtctcaccatcatcaccaccaccaccattga